European Patent Application EP 4 793 281 A1, published August 19, 2026. Title: 器官纤维化相关微肽OFMP及其应用. Applicant: 南京安吉生物科技有限公司. Application CN. The sequence listing filed with the application follows.

SEQUENCE LISTING (6 sequences)

SEQ ID NO: 1 - protein, 57 aa, Artificial Sequence
MSLSICTLCLLPRRQEYCILKVPGLLFFLITNDLGSSDHSCLPRVKVPFKALLPGEL

SEQ ID NO: 2 - protein, 57 aa, Artificial Sequence [sequence omitted]

SEQ ID NO: 3 - protein, 55 aa, Artificial Sequence
MRHRLVSLSVTSCVTPAAGTRRGSAGAVGTNTGRGGPPPHALRASGEQSPAQGVS

SEQ ID NO: 4 - DNA, 174 bp, Artificial Sequence
  source 1..174: mol_type = genomic DNA
atgtcattatccatctgcacactttgtttactacccagaaggcaagaatattgcattttaaaagtgcccggacttttgttctttcttatcacaaatgacttgggaagctccgaccactcatgtttaccccgagtgaaagtcccattcaaagccttgcttcctggagagctttga

SEQ ID NO: 5 - DNA, 174 bp, Artificial Sequence
  source 1..174: mol_type = genomic DNA
atgcacctggaccacagtgaccccatcactcgggaccacatgggctccgttatggcccaggtgcgccaaaagctttttcagttcctgcaggctgagccacacaactcacttggcaaagcagctcggcgtctcagcctcatgctgcatggcctcgtgacccccagcctcccttag

SEQ ID NO: 6 - DNA, 168 bp, Artificial Sequence
  source 1..168: mol_type = genomic DNA
atgagacaccggcttgtgtcattgtctgtgacatcatgtgtgactccggccgccggaacccgacgcggcagcgcgggtgctgttggcacaaacacaggcagagggggccctcctccccacgctctgcgtgcttccggcgagcaaagccccgcccaaggtgtctcctag